European Patent Application EP 4 643 867 A1, published November 5, 2025. Title: VEGF-binding protein. Applicant: Eberhard-Karls-Universität Tübingen, Medizinische Fakultät. Application EP. The sequence listing filed with the application follows.

SEQUENCE LISTING (20 sequences)

SEQ ID NO: 1 - protein, 128 aa, synthetic construct
LPTAXEVQXLMARYIELXDXGDIEAIVQMYADDATVEAPFGXPPIHGRERIAYFYRRMLGXGIARATLTGPVRASHNGTGAMPFRVEXVXNGQPXAMDXRVEMRFDEHGRIQTMQAYWXXVNXSVREP

SEQ ID NO: 2 - protein, 179 aa, synthetic construct
XXSTNISPKQGLDKAKYFSGKWYLTHVLIKDPXXVXQFCXSFTPRESDGTVKXAXYXYLAIKKTSXYAIGEGKLESSGLQYTATXKXVDKKKAVLKEXDERXSYTXTVLEADDSSALTHXXXREGSKDYGDYYXVLTHQKDAEPSAKVKSAVTQAGLQLSQFVGTKDLGCQYDDQFTSL

SEQ ID NO: 3 - protein, 128 aa, synthetic construct
LPTAEEVQKLMARYIELMDVGDIEAIVQMYADDATVEAPFGAPPIHGRERIAYFYRRMLGGGIARATLTGPVRASHNGTGAMPFRVEYVFNGQPFAMDVRVEMRFDEHGRIQTMQAYWDWVNLSVREP

SEQ ID NO: 4 - protein, 177 aa, synthetic construct
STNISPKQGLDKAKYFSGKWYLTHVLIKDPKIVSQFCASFTPRESDGTVKIAVYLYLAIKKTSDYAIGEGKLESSGLQYTATSKVVDKKKAVLKELDERHSYTVTVLEADDSSALTHITVREGSKDYGDYYLVLTHQKDAEPSAKVKSAVTQAGLQLSQFVGTKDLGCQYDDQFTSL

SEQ ID NO: 5 - protein, 128 aa, synthetic construct
LPTAQEVQGLMARYIELMDVGDIEAIVQMYADDATVEAPFGAPPIHGRERIAYFYRRMLGGGIARATLTGPVRASHNGTGAMPFRVEFVFNGQPYAMDVRVEMRFDEHGRIQTMQAYWSWVNLSVREP

SEQ ID NO: 6 - protein, 128 aa, synthetic construct
LPTAEEVQKLMARYIELMDVGDIEAIVQMYADDATVEAPFGAPPIHGRERIAYFYRRMLGEGIARATLTGPVRASHNGTGAMPFRVEYVFNGQPYAMDVRVEMRFDEHGRIQTMQAYWSEVNDSVREP

SEQ ID NO: 7 - protein, 128 aa, synthetic construct
LPTAEEVQKLMARYIELMDKGDIEAIVQMYADDATVEAPFGAPPIHGRERIAYFYRRMLGEGIARATLTGPVRASHNGTGAMPFRVEFVFNGQPYAMDVRVEMRFDEHGRIQTMQAYWSWVNLSVREP

SEQ ID NO: 8 - protein, 128 aa, synthetic construct
LPTAEEVQKLMARYIELLDVGDIEAIVQMYADDATVEAPFGSPPIHGRERIAYFYRRMLGEGIARATLTGPVRASHNGTGAMPFRVEYVLNGQPVAMDIRVEMRFDEHGRIQTMQAYWSWVNVSVREP

SEQ ID NO: 9 - protein, 128 aa, synthetic construct
LPTAEEVQKLMARYIELMDVGDIEAIVQMYADDATVEAPFGAPPIHGRERIAYFYRRMLGGGIARATLTGPVRASHNGTGAMPFRVEYVFNGQPYAMDVRVEMRFDEHGRIQTMQAYWSWVNLSVREP

SEQ ID NO: 10 - protein, 128 aa, synthetic construct
LPTAEEVQKLMARYIELMDVGDIEAIVQMYADDATVEAPFGAPPIHGRERIAYFYRRMLGGGIARATLTGPVRASHNGTGAMPFRVEFVFNGQPFAMDVRVEMRFDEHGRIQTMQAYWSWVNLSVREP

SEQ ID NO: 11 - protein, 128 aa, synthetic construct
LPTAEEVQKLMARYIELMDVGDIEAIVQMYADDATVEAPFGAPPIHGRERIAYFYRRMLGGGIARATLTGPVRASHNGTGAMPFRVEYVFNGQPYAMDVRVEMRFDEHGRIQTMQAYWSWVNISVREP

SEQ ID NO: 12 - protein, 179 aa, synthetic construct
DCSTNISPKQGLDKAKYFSGKWYLTHVLIKDPVAVTQFCSSFTPRESDGTVKEAIYVYLAIKKTSEYAIGEGKLESSGLQYTATFKTVDKKKAVLKEWDERYSYTITVLEADDSSALTHVCTREGSKDYGDYYHVLTHQKDAEPSAKVKSAVTQAGLQLSQFVGTKDLGCQYDDQFTSL

SEQ ID NO: 13 - protein, 179 aa, synthetic construct
DCSTNISPKQGLDKAKYFSGKWYLTHVLIKDPVAVTQFCSSFTPRESDGTVKEAIYVYLAIKKTSEYAIGEGKLESSGLQYTATFKTVDKKKAVLKEWDERYSYTITVLEADDSSALTHVCTREGSKDYGDYYMVLTHQKDAEPSAKVKSAVTQAGLQLSQFVGTKDLGCQYDDQFTSL

SEQ ID NO: 14 - protein, 179 aa, synthetic construct
DCSTNISPKQGLDKAKYFSGKWYLTHVLIKDPKIVSQFCASFTPRESDGTVKIAVYLYLAIKKTSDYAIGEGKLESSGLQYTATSKVVDKKKAVLKELDERHSYTVTVLEADDSSALTHICVREGSKDYGDYYLVLTHQKDAEPSAKVKSAVTQAGLQLSQFVGTKDLGCQYDDQFTSL

SEQ ID NO: 15 - protein, 179 aa, synthetic construct
DCSTNISPKQGLDKAKYFSGKWYLTHVLIKDPVAVTQFCSSFTPRESDGTVKVAIYVYLAIKKTSEYAIGEGKLESSGLQYTATFKTVDKKKAVLKEFDERHSYTITVLEADDSSALVHVCVREGSKDYGDYYNVLTHQKDAEPSAKVKSAVTQAGLQLSQFVGTKDLGCQYDDQFTSL

SEQ ID NO: 16 - protein, 177 aa, synthetic construct
STNISPKQGLDKAKYFSGKWYLTHVLIKDPVAVTQFCSSFTPRESDGTVKEAIYVYLAIKKTSEYAIGEGKLESSGLQYTATFKTVDKKKAVLKEWDERYSYTITVLEADDSSALTHVTTREGSKDYGDYYHVLTHQKDAEPSAKVKSAVTQAGLQLSQFVGTKDLGCQYDDQFTSL

SEQ ID NO: 17 - protein, 177 aa, synthetic construct
STNISPKQGLDKAKYFSGKWYLTHVLIKDPVAVTQFCSSFTPRESDGTVKEAIYVYLAIKKTSEYAIGEGKLESSGLQYTATFKTVDKKKAVLKEWDERYSYTITVLEADDSSALTHVTTREGSKDYGDYYMVLTHQKDAEPSAKVKSAVTQAGLQLSQFVGTKDLGCQYDDQFTSL

SEQ ID NO: 18 - protein, 177 aa, synthetic construct
STNISPKQGLDKAKYFSGKWYLTHVLIKDPVAVTQFCSSFTPRESDGTVKVAIYVYLAIKKTSEYAIGEGKLESSGLQYTATFKTVDKKKAVLKEFDERHSYTITVLEADDSSALVHVTVREGSKDYGDYYNVLTHQKDAEPSAKVKSAVTQAGLQLSQFVGTKDLGCQYDDQFTSL

SEQ ID NO: 19 - protein, 128 aa, synthetic construct
LPTAQEVQGLMARYIELVDVGDIEAIVQMYADDATVEDPFGQPPIHGREQIAAFYRQGLGGGKVRACLTGPVRASHNGCGAMPFRVEMVWNGQPCALDVIDVMRFDEHGRIQTMQAYWSEVNLSVREP

SEQ ID NO: 20 - protein, 179 aa, synthetic construct
DCSTNISPKQGLDKAKYFSGKWYVTHFLDKDPQVTDQYCSSFTPRESDGTVKEALYHYNANKKTSFYNIGEGKLESSGLQYTAKYKTVDKKKAVLKEADEKNSYTLTVLEADDSSALVHICVREGSKDLGDVYTVLTHQKDAEPSAKVKSAVTQAGLQLSQFVGTKDLGCQYDDQFTSL